European Patent Application EP 4 650 448 A1, published November 19, 2025. Title: 一种基于RNA核酶的DEAR核酸操纵系统及其应用. Applicant: 清华大学. The sequence listing filed with the application follows.

SEQUENCE LISTING (58 sequences)

SEQ ID NO: 1 - RNA, 633 nt, synthetic construct
  source 1..633: mol_type = other RNA
  misc_feature 181..186: note = n=a, u, g, or c
gtgcgctcggcatgggtgcaatctctagggtgaaagtcccgaactgcgaaggcagaagtagcagttagcttaacgcaagggtgtccgtggtgacgcggaatctgaaggaagcgggcggcaaacttccggtctgaggaacacgaacttcatataaggctaggtatcattggatgagtttgcnnnnnnaaacaaagtcctttctgccgaaggtgatacagagtaaatgaagcagatagatggaaggaaagattgtactcttacccgaggaggtctgatggatacgtgaagtgcgcttcataacctacttagtgataagtaactgaaccatcagaagtcagcagaggtcatagtacgaatcggtctagaacgattcggaaggactgaacaatcaagagaaaatagcccttggcattcagtacgtcatgatgaacacagaaaacatggtacctcccaagagaaaggaaacggtgaatcccgtgggaatcttttggagggtggagtgacgactggcataagaagatcagctatttacggaaggaagcttgcgtcattatcttgattgaaccgccgtatacggaaccgtacgtacggtggtgtgagaggacggaggttaatcacctcctcctactcgat

SEQ ID NO: 2 - RNA, 621 nt, synthetic construct
  source 1..621: mol_type = other RNA
  misc_feature 181..186: note = n=a, u, g, or c
gtacgacgggcatgtcgtacatctgaggtgcaagtcctctgtggacacctgctaccggtgaacccaatagcgactcccaagcctgactatcgcgaggtaacggggagaggaagggatagcgaaatcgtggctctacgaacagaaacgtgatattaaggcgtatatagtggatgagggggcnnnnnnctctaaagtccaaaaaggtagtcgtaatctatgtgcgtaaatcacgagagtaaacgaggaaagatgtacgacttatcccgtgaggtctcatgagcgtcaagtagacgtagtaataacgaatcatgagaagtcagccgaggtcatagtagtgatgaagtttctgtaatggaaacggagcgaaggaccgaacgattaaatgataccctatctaactgattttgtctgccctaacacctggtctgaaatgacggtactcgcagaacgtatgctgaaagaggctgctcacaaatataggacggcacaagcggaacgaaatcatatataggtaggtgtgggaacaaaaaaagtgttctcgccaaagtttagttgaaccgccgtgtgccgaacggcacgcacggtggtgtgagagggactatcaattagtccctactcgat

SEQ ID NO: 3 - RNA, 647 nt, synthetic construct
  source 1..647: mol_type = other RNA
  misc_feature 181..186: note = n=a, u, g, or c
gtatgcccggcatgggcgatagctttagggtgaaagtcccgaacaggggttggcaacaccaactgttagccaagagcaagggtgtccatcgtgaggtggaatctgaaagaagctggaggcaaattcccgacctgaggtacacgaatcacattcgaggctgttatattcgggcaagactgcnnnnnnagtcaaagccctatgttgccaagggatatagcagtaaatgtggcaggtacatgggatgaaagttatcgctcttatccggggaggtctgtcgatccggtaatggtaaggaagtccttaacaataccaacccgcatcgtgaggtgtcggctgagtcggcagaagtcagcagaggccatagtactcctaacgaggaagggccgaaggtcagggcagactaagaacggtgcgttcgagagaatttgctgatagcagttgtctctgaaacagagacctatctataagagggagtggtgaagccacaatggcttatagaagggctgagaattctccggcacaatacccgaaaatcttaatcttaatcgctgagtaatcagttaaccctggccaaccgccggatgcggacccgcatgtccggtggtgtgggagggtcggcggagattatctccgccccctatcccaat

SEQ ID NO: 4 - RNA, 650 nt, synthetic construct
  source 1..650: mol_type = other RNA
  misc_feature 179..184: note = n=a, u, g, or c
gtgcgcccagcatgggcgcaatcttggaggtgaaagtcctcccgtaagttgatcacagcgaacgaagcgaagcgcaactgcatgagggcgactgagtgtggggaggaagcgtggagcgaagctgcgagccgatgaacaagaatcggatagaaggcggtgccgaccagggcgagcgggcnnnnnnccgcgaagctctcgtgatcaagggtcaggcggcgtagatccggcggttgtgcagtgaaggattgcgttcttacctggggagatctcgctttgtgcctgaaagggcgacggtgtaagccggagcgagaagtcagcagaggtcgtagtagttggcggcatggccggagaggctggaagctgttggcgaaggaccaaaggagcagaagggcaagtctgcctgaccatccgaaatggatatgcttcagatgcccggatacggggctcgttacgaaaagtgcagcaggtgaagcctgaaatacttgtgacagcgaagaaccagatcggccgggttggggacaggcgagtccaggcgtcatgttcgggtatgggcatgacgacctcaaccgtttcaaccgcccggtgcggacccgcatgccgggtggtgtggcaggggaccggtcagttatactgaccgcccctatgccgat

SEQ ID NO: 5 - RNA, 640 nt, synthetic construct
  source 1..640: mol_type = other RNA
  misc_feature 181..186: note = n=a, u, g, or c
gtgcgcccggcatgtacatgaactatagggtgtaagtcccgaaccccgaagacagaagtagaggttagccaagagcaagggtgtccgtggtgacgcggaatctgaaggaagctggaggcaaaacaccggtccgaggaacacgaacctcatataaggctaggtatgattgagtgagtttgcnnnnnnaaacaaagctctttctgtcgaaggtcatatcgagtaaatgaggcggatagatggtgtgaaagtgcatgtacttacccggggaggtctggcggatatgtgaagtactcttcataacctacttagtgataagtagctgaaccgtcagaagtcagcagaggtcatagtattagttggtctagaacaactaagaaggaccgaacaattaagagagaatagcccttggtattcagtgagtcatgatgaacacagaaaacgtagtacctcacttgagggaggaagcggtgaatcccgtgggagacctcttggagggtggagtgaccactggcataaagagaacagctattcacggaagttataaagacttgcgtcaattatcttaattgaaccgccgtatacggaaccgtacgtacggtggtgtgagaggacgggagttaatcgctccctcctactcgat

SEQ ID NO: 6 - RNA, 595 nt, synthetic construct
  source 1..595: mol_type = other RNA
  misc_feature 214..219: note = note = n=a, u, g, or c
gtgtgcccagtatgggcatcttttgttttaccgaaaggtaaaatattaatctagagggtgcaagtcccttatgggcaggggtaacgccttgaaccattagtaagccgcaagggtggtgatcgtgaggtcacatctgaagaaagcgggactacaaaacccggtactgacgaacaggaaccgtatacagaggcatttatgcatgggtaagcaaccnnnnnnttgtaaagccctaagaataccaaaagtgcatttatgtagatacggcagggatcgggggaaagaagatgctcttacctggggaggtctccagtaccacgtgtttgtacaggagaagtcagcagaggtcatagtacctaagggaaacgagttgcagcgaaactgcataggtctcacaattaggaaaggaccgaacgtaatcctcttcaaaattcgcataggaacacaacttgtgtagcctatgcttaaactagaagatagtgccaagggtgaaaagagctttggtgtgatggtttacgaaccgccgtatacgagacccgtacgtgcggtggtgtgaggggtgcacttcgtcatttgatggcggagccatccactcgat

SEQ ID NO: 7 - RNA, 644 nt, synthetic construct
  source 1..644: mol_type = other RNA
  misc_feature 206..211: note = n=a, u, g, or c
gtgtgccctgaatggcaaatatagttctttcaaatagaataatccagagagtgaaagtctcttatgcgcctcttaaattgaggaagcattagcaagtcgcaaggtggtttgtcgtgagatatgcactgaagtaagcgagactgcaaaggtcggtactgacgtacagaaactgtatatagaggcatgatgaatcgggtgaggtagcnnnnnntactaaagccccaagattacaaaccattcatcatgtagatgcagcagcgattgaccgaaggatatttgtcttaccgggggaggtctgttgataggttgactaagattggcgcgacaatcgaagcaacaattcccgaaagcaatagggagtttcaatagaagtcagcagaggtcatagtagttggtagttacgagccgaagataaatcggacggtctcacaagccagcgaaggactgaatgttaagtcgtttctaatgcaataaggagctttaagcttcgcgcttagcagccttgttataaaagaaacaaagtgcaattggtgaaaagagcgattgtactcatgcttaacaaaccgccgtgtacgagacccatacgcacggtggtgtgaggggcactccccacctgttcattcaggtggggctgtccactcgat

SEQ ID NO: 8 - RNA, 636 nt, synthetic construct
  source 1..636: mol_type = other RNA
  misc_feature 180..185: note = n=a, u, g, or c
gtgcgcccagcatgtgcaatagctaagcggtgaaagtccgttgtgggccaggtagcgggaaccactagtcgaaggcaagggtgtccatcgtgaggtggaatctgaaggaagcccaaggcaaagtcccggtccgatgaacaagaaccagatataaggctaagtgaagtggacgagtttgcnnnnnnaaacgaagtccaacagctaccctgaacttcacggagtagatctggcggatagatgggatgaaagttattgcacttacctggggagatctcaagaatatgctattgaggcaacccatacagcaatgtatggctgaatcttgagaagtcagcagaagtcatagtactcattgagagatgaggaaggactgaacaacagaaggtttcgaatcttgaaagatgcgaagggatacggaaaaggcatacaacttcgactagaaggtttcctacatgaagataagggagagcccgaaaataatgtaccaagcgcctagtataacttctacatctgaaagagggagaaacgatgtgaagggtcttatacatcaaacctgttgaaccgccgtatacagaatggtacgtacggtggtgcggaaggacggcagataaattaattatctacctcctactcgat

SEQ ID NO: 9 - RNA, 451 nt, synthetic construct
  source 1..451: mol_type = other RNA
  misc_feature 181..186: note = n=a, u, g, or c
gtgcgcccggcatgcgtatgaactatagggtgcaagtcccgaaccccgaagacagaagtagaggttagccaagagcaagggtgtccgtggcgacgcggaatctgaaggaagctggaggcaaaacaccggtccgaggaacacgaatctcatataaggctaggtatgattggatgagtttgcnnnnnnaaacaaagtcctttctgtcgaaggtcatatcgagtaaatgaggcggatagatggtgtgaaagtgcatacgcttacccggggaggtctgatggaaacgtgaagtacccttcataacctacttggtgacaagtagctgaaccatcagaagtcagcagaggtcatagtacgaaactttgcgttattcatcttaattgaaccgccgtatacggaaccgtacgtacggtggtgtgagaggtcgggagttaatcactccctcctactcgat

SEQ ID NO: 10 - RNA, 633 nt, Anoxybacillus pushchinoensis
  source 1..633: mol_type = genomic RNA
gtgcgctcggcatgggtgcaatctctagggtgaaagtcccgaactgcgaaggcagaagtagcagttagcttaacgcaagggtgtccgtggtgacgcggaatctgaaggaagcgggcggcaaacttccggtctgaggaacacgaacttcatataaggctaggtatcattggatgagtttgcaagacaaaacaaagtcctttctgccgaaggtgatacagagtaaatgaagcagatagatggaaggaaagattgtactcttacccgaggaggtctgatggatacgtgaagtgcgcttcataacctacttagtgataagtaactgaaccatcagaagtcagcagaggtcatagtacgaatcggtctagaacgattcggaaggactgaacaatcaagagaaaatagcccttggcattcagtacgtcatgatgaacacagaaaacatggtacctcccaagagaaaggaaacggtgaatcccgtgggaatcttttggagggtggagtgacgactggcataagaagatcagctatttacggaaggaagcttgcgtcattatcttgattgaaccgccgtatacggaaccgtacgtacggtggtgtgagaggacggaggttaatcacctcctcctactcgat

SEQ ID NO: 11 - RNA, 621 nt, Streptococcus azizii
  source 1..621: mol_type = genomic RNA
gtacgacgggcatgtcgtacatctgaggtgcaagtcctctgtggacacctgctaccggtgaacccaatagcgactcccaagcctgactatcgcgaggtaacggggagaggaagggatagcgaaatcgtggctctacgaacagaaacgtgatattaaggcgtatatagtggatgagggggctaggcactctaaagtccaaaaaggtagtcgtaatctatgtgcgtaaatcacgagagtaaacgaggaaagatgtacgacttatcccgtgaggtctcatgagcgtcaagtagacgtagtaataacgaatcatgagaagtcagccgaggtcatagtagtgatgaagtttctgtaatggaaacggagcgaaggaccgaacgattaaatgataccctatctaactgattttgtctgccctaacacctggtctgaaatgacggtactcgcagaacgtatgctgaaagaggctgctcacaaatataggacggcacaagcggaacgaaatcatatataggtaggtgtgggaacaaaaaaagtgttctcgccaaagtttagttgaaccgccgtgtgccgaacggcacgcacggtggtgtgagagggactatcaattagtccctactcgat

SEQ ID NO: 12 - RNA, 647 nt, Desulfotomaculum_H ferrireducens
  source 1..647: mol_type = genomic RNA
gtatgcccggcatgggcgatagctttagggtgaaagtcccgaacaggggttggcaacaccaactgttagccaagagcaagggtgtccatcgtgaggtggaatctgaaagaagctggaggcaaattcccgacctgaggtacacgaatcacattcgaggctgttatattcgggcaagactgccagacaagtcaaagccctatgttgccaagggatatagcagtaaatgtggcaggtacatgggatgaaagttatcgctcttatccggggaggtctgtcgatccggtaatggtaaggaagtccttaacaataccaacccgcatcgtgaggtgtcggctgagtcggcagaagtcagcagaggccatagtactcctaacgaggaagggccgaaggtcagggcagactaagaacggtgcgttcgagagaatttgctgatagcagttgtctctgaaacagagacctatctataagagggagtggtgaagccacaatggcttatagaagggctgagaattctccggcacaatacccgaaaatcttaatcttaatcgctgagtaatcagttaaccctggccaaccgccggatgcggacccgcatgtccggtggtgtgggagggtcggcggagattatctccgccccctatcccaat

SEQ ID NO: 13 - RNA, 650 nt, Collimonas pratensis
  source 1..650: mol_type = genomic RNA
gtgcgcccagcatgggcgcaatcttggaggtgaaagtcctcccgtaagttgatcacagcgaacgaagcgaagcgcaactgcatgagggcgactgagtgtggggaggaagcgtggagcgaagctgcgagccgatgaacaagaatcggatagaaggcggtgccgaccagggcgagcgggcaatgaaccgcgaagctctcgtgatcaagggtcaggcggcgtagatccggcggttgtgcagtgaaggattgcgttcttacctggggagatctcgctttgtgcctgaaagggcgacggtgtaagccggagcgagaagtcagcagaggtcgtagtagttggcggcatggccggagaggctggaagctgttggcgaaggaccaaaggagcagaagggcaagtctgcctgaccatccgaaatggatatgcttcagatgcccggatacggggctcgttacgaaaagtgcagcaggtgaagcctgaaatacttgtgacagcgaagaaccagatcggccgggttggggacaggcgagtccaggcgtcatgttcgggtatgggcatgacgacctcaaccgtttcaaccgcccggtgcggacccgcatgccgggtggtgtggcaggggaccggtcagttatactgaccgcccctatgccgat

SEQ ID NO: 14 - RNA, 640 nt, Bacillus_O smithii
  source 1..640: mol_type = genomic RNA
gtgcgcccggcatgtacatgaactatagggtgtaagtcccgaaccccgaagacagaagtagaggttagccaagagcaagggtgtccgtggtgacgcggaatctgaaggaagctggaggcaaaacaccggtccgaggaacacgaacctcatataaggctaggtatgattgagtgagtttgcataacaaaacaaagctctttctgtcgaaggtcatatcgagtaaatgaggcggatagatggtgtgaaagtgcatgtacttacccggggaggtctggcggatatgtgaagtactcttcataacctacttagtgataagtagctgaaccgtcagaagtcagcagaggtcatagtattagttggtctagaacaactaagaaggaccgaacaattaagagagaatagcccttggtattcagtgagtcatgatgaacacagaaaacgtagtacctcacttgagggaggaagcggtgaatcccgtgggagacctcttggagggtggagtgaccactggcataaagagaacagctattcacggaagttataaagacttgcgtcaattatcttaattgaaccgccgtatacggaaccgtacgtacggtggtgtgagaggacgggagttaatcgctccctcctactcgat

SEQ ID NO: 15 - RNA, 595 nt, Leeuwenhoekiella
  source 1..595: mol_type = genomic RNA
gtgtgcccagtatgggcatcttttgttttaccgaaaggtaaaatattaatctagagggtgcaagtcccttatgggcaggggtaacgccttgaaccattagtaagccgcaagggtggtgatcgtgaggtcacatctgaagaaagcgggactacaaaacccggtactgacgaacaggaaccgtatacagaggcatttatgcatgggtaagcaaccacatcattgtaaagccctaagaataccaaaagtgcatttatgtagatacggcagggatcgggggaaagaagatgctcttacctggggaggtctccagtaccacgtgtttgtacaggagaagtcagcagaggtcatagtacctaagggaaacgagttgcagcgaaactgcataggtctcacaattaggaaaggaccgaacgtaatcctcttcaaaattcgcataggaacacaacttgtgtagcctatgcttaaactagaagatagtgccaagggtgaaaagagctttggtgtgatggtttacgaaccgccgtatacgagacccgtacgtgcggtggtgtgaggggtgcacttcgtcatttgatggcggagccatccactcgat

SEQ ID NO: 16 - RNA, 644 nt, PALSA-967 sp003151745
  source 1..644: mol_type = genomic RNA
gtgtgccctgaatggcaaatatagttctttcaaatagaataatccagagagtgaaagtctcttatgcgcctcttaaattgaggaagcattagcaagtcgcaaggtggtttgtcgtgagatatgcactgaagtaagcgagactgcaaaggtcggtactgacgtacagaaactgtatatagaggcatgatgaatcgggtgaggtagcacatcatactaaagccccaagattacaaaccattcatcatgtagatgcagcagcgattgaccgaaggatatttgtcttaccgggggaggtctgttgataggttgactaagattggcgcgacaatcgaagcaacaattcccgaaagcaatagggagtttcaatagaagtcagcagaggtcatagtagttggtagttacgagccgaagataaatcggacggtctcacaagccagcgaaggactgaatgttaagtcgtttctaatgcaataaggagctttaagcttcgcgcttagcagccttgttataaaagaaacaaagtgcaattggtgaaaagagcgattgtactcatgcttaacaaaccgccgtgtacgagacccatacgcacggtggtgtgaggggcactccccacctgttcattcaggtggggctgtccactcgat

SEQ ID NO: 17 - RNA, 636 nt, Petrotoga mobilis
  source 1..636: mol_type = genomic RNA
gtgcgcccagcatgtgcaatagctaagcggtgaaagtccgttgtgggccaggtagcgggaaccactagtcgaaggcaagggtgtccatcgtgaggtggaatctgaaggaagcccaaggcaaagtcccggtccgatgaacaagaaccagatataaggctaagtgaagtggacgagtttgccactcaaaacgaagtccaacagctaccctgaacttcacggagtagatctggcggatagatgggatgaaagttattgcacttacctggggagatctcaagaatatgctattgaggcaacccatacagcaatgtatggctgaatcttgagaagtcagcagaagtcatagtactcattgagagatgaggaaggactgaacaacagaaggtttcgaatcttgaaagatgcgaagggatacggaaaaggcatacaacttcgactagaaggtttcctacatgaagataagggagagcccgaaaataatgtaccaagcgcctagtataacttctacatctgaaagagggagaaacgatgtgaagggtcttatacatcaaacctgttgaaccgccgtatacagaatggtacgtacggtggtgcggaaggacggcagataaattaattatctacctcctactcgat

SEQ ID NO: 18 - RNA, 451 nt, Lysinibacillus sphaericus_B
  source 1..451: mol_type = genomic RNA
gtgcgcccggcatgcgtatgaactatagggtgcaagtcccgaaccccgaagacagaagtagaggttagccaagagcaagggtgtccgtggcgacgcggaatctgaaggaagctggaggcaaaacaccggtccgaggaacacgaatctcatataaggctaggtatgattggatgagtttgcattacaaaacaaagtcctttctgtcgaaggtcatatcgagtaaatgaggcggatagatggtgtgaaagtgcatacgcttacccggggaggtctgatggaaacgtgaagtacccttcataacctacttggtgacaagtagctgaaccatcagaagtcagcagaggtcatagtacgaaactttgcgttattcatcttaattgaaccgccgtatacggaaccgtacgtacggtggtgtgagaggtcgggagttaatcactccctcctactcgat

SEQ ID NO: 19 - DNA, 17 bp, synthetic construct
  source 1..17: mol_type = other DNA
taatacgactcactata

SEQ ID NO: 20 - RNA, 24 nt, synthetic construct
  source 1..24: mol_type = other RNA
accaaatgtcttagcggatcggat

SEQ ID NO: 21 - RNA, 24 nt, synthetic construct
  source 1..24: mol_type = other RNA
gagaaatgcctacaacacaccacc

SEQ ID NO: 22 - RNA, 24 nt, synthetic construct
  source 1..24: mol_type = other RNA
gtaacatgtctgcaaaacctccaa

SEQ ID NO: 23 - RNA, 24 nt, synthetic construct
  source 1..24: mol_type = other RNA
ggaggcttcattaacggcaacaga

SEQ ID NO: 24 - RNA, 24 nt, synthetic construct
  source 1..24: mol_type = other RNA
acccactgttatccgacgacgagc

SEQ ID NO: 25 - RNA, 24 nt, synthetic construct
  source 1..24: mol_type = other RNA
cttcactgatgtacaaccaagaga

SEQ ID NO: 26 - DNA, 1029 bp, synthetic construct
  source 1..1029: mol_type = other DNA
atgggtaaaaagcctgaactcaccgcgacgtctgtcgagaagtttctgatcgaaaagttcgacagcgtttccgacctgatgcagctctcggagggcgaagaatctcgtgctttcagcttcgatgtaggagggcgtggatatgtcctgcgggtaaatagctgcgccgatggtttctacaaagatcgttatgtttatcggcactttgcatcggccgcgctcccgattccggaagtgcttgacattggggaattcagcgagagcctgacctattgcatctcccgccgtgcacagggtgtcacgttgcaagacctgcctgaaaccgaactgcccgctgttctgcagccggtcgcggaggcaatggatgcgatcgctgcggccgatcttagccagacgagcgggttcggcccattcggaccgcaaggaatcggtcaatacactacatggcgtgatttcatatgcgcgattgctgatccccatgtgtatcactggcaaactgtgatggacgacaccgtcagtgcgtccgtcgcgcaggctctcgatgagctgatgctttgggccgaggactgccccgaagtccggcacctcgtgcacgcggatttcggctccaacaatgtcctgacggacaatggccgcataacagcggtcattgactggagcgaggcgatgttcggggattcccaatacgaggtcgccaacatcttcttctggaggccgtggttggcttgtatggagcagcagacgcgctacttcgagcggaggcatccggagcttgcaggatcgccgcggctccgggcgtatatgctccgcattggtcttgaccaactctatcagagcttggttgacggcaatttcgatgatgcagcttgggcgcagggtcgatgcgacgcaatcgtccgatccggagccgggactgtcgggcgtacacaaatcgcccgcagaagcgcggccgtctggaccgatggctgtgtagaagtactcgccgatagtggaaaccgacgccccagcactcgtccgagggcaaaggaataa

SEQ ID NO: 27 - RNA, 24 nt, synthetic construct
  source 1..24: mol_type = other RNA
gtaacatgagtgcaaaacctccaa

SEQ ID NO: 28 - RNA, 24 nt, synthetic construct
  source 1..24: mol_type = other RNA
acccactgtaatccgacgacgagc

SEQ ID NO: 29 - DNA, 60 bp, synthetic construct
  source 1..60: mol_type = other DNA
tagagaactttgtctttgtctttgtctttgtctttgtctttttactgggtagtgcgtagg

SEQ ID NO: 30 - DNA, 60 bp, synthetic construct
  source 1..60: mol_type = other DNA
tagagaactttgcctatgcctatgcctatgcctatgcctatttactgggtagtgcgtagg

SEQ ID NO: 31 - DNA, 60 bp, synthetic construct
  source 1..60: mol_type = other DNA
tagagaactttgtctgtgtctgtgtctgtgtctgtgtctgtttactgggtagtgcgtagg

SEQ ID NO: 32 - DNA, 60 bp, synthetic construct
  source 1..60: mol_type = other DNA
tagagaacttttcattttcattttcattttcattttcatttttactgggtagtgcgtagg

SEQ ID NO: 33 - DNA, 60 bp, synthetic construct
  source 1..60: mol_type = other DNA
tagagaactttgttattgttattgttattgttattgttattttactgggtagtgcgtagg

SEQ ID NO: 34 - DNA, 60 bp, synthetic construct
  source 1..60: mol_type = other DNA
tagagaactttgatgttgatgttgatgttgatgttgatgttttactgggtagtgcgtagg

SEQ ID NO: 35 - DNA, 24 bp, synthetic construct
  source 1..24: mol_type = other DNA
accaaatgtcttagcggatcggat

SEQ ID NO: 36 - DNA, 24 bp, synthetic construct
  source 1..24: mol_type = other DNA
gagaaatgcctacaacacaccacc

SEQ ID NO: 37 - DNA, 24 bp, synthetic construct
  source 1..24: mol_type = other DNA
gtaacatgtctgcaaaacctccaa

SEQ ID NO: 38 - DNA, 24 bp, synthetic construct
  source 1..24: mol_type = other DNA
ggaggcttcattaacggcaacaga

SEQ ID NO: 39 - DNA, 24 bp, synthetic construct
  source 1..24: mol_type = other DNA
acccactgttatccgacgacgagc

SEQ ID NO: 40 - DNA, 24 bp, synthetic construct
  source 1..24: mol_type = other DNA
cttcactgatgtacaaccaagaga

SEQ ID NO: 41 - DNA, 12 bp, synthetic construct
  source 1..12: mol_type = other DNA
tgtcttaagaca

SEQ ID NO: 42 - DNA, 35 bp, synthetic construct
  source 1..35: mol_type = other DNA
ttgacagctagctcagtcctaggtataatactagt

SEQ ID NO: 43 - DNA, 30 bp, synthetic construct
  source 1..30: mol_type = other DNA
ttgacaattaatcatccggctcgtataatg

SEQ ID NO: 44 - DNA, 20 bp, synthetic construct
  source 1..20: mol_type = other DNA
gcgataagtcgtgtcttacc

SEQ ID NO: 45 - DNA, 32 bp, synthetic construct
  source 1..32: mol_type = other DNA
ggatgagtttgcaaacaaagtcctttctgccg

SEQ ID NO: 46 - DNA, 37 bp, synthetic construct
  source 1..37: mol_type = other DNA
aggactttgtttgcaaactcatccaatgatacctagc

SEQ ID NO: 47 - DNA, 39 bp, synthetic construct
  source 1..39: mol_type = other DNA
agtacagcatcggcctggccatcggcaccaactctgtgg

SEQ ID NO: 48 - DNA, 40 bp, synthetic construct
  source 1..40: mol_type = other DNA
ggccaggccgatgctgtacttcttgtcagaaccgtggtga

SEQ ID NO: 49 - DNA, 39 bp, synthetic construct
  source 1..39: mol_type = other DNA
ccgactacgatgtggacgccatcgtgcctcagagctttc

SEQ ID NO: 50 - DNA, 37 bp, synthetic construct
  source 1..37: mol_type = other DNA
ggcgtccacatcgtagtcggacagccggttgatgtcc

SEQ ID NO: 51 - DNA, 24 bp, synthetic construct
  source 1..24: mol_type = other DNA
accaaactatcgagcggatcggat

SEQ ID NO: 52 - DNA, 763 bp, synthetic construct
  source 1..763: mol_type = other DNA
gctagcgccaccatgtccggtagcggtggctcaagcggaagctgtcttaagacattcttgcggaagtgggtctggctcaggaggtgtcttaagacagtccggttcaagtggaagttcaagtggaagtgtcttaagacattcttgtggaggttcctctggtagtaccgagtacaagcccacggtgcgcctcgccacccgcgacgacgtccccagggccgtacgcaccctcgccgccgcgttcgccgactaccccgccacgcgccacaccgtcgatccggaccgccacatcgagcgggtcaccgagctgcaagaactcttcctcacgcgcgtcgggctcgacatcggcaaggtgtgggtcgcggacgacggcgccgcggtggcggtctggaccacgccggagagcgtcgaagcgggggcggtgttcgccgagatcggcccgcgcatggccgagttgagcggttcccggctggccgcgcagcaacagatggaaggcctcctggcgccgcaccggcccaaggagcccgcgtggttcctggccaccgtcggagtctcgcccgaccaccagggcaagggtctgggcagcgccgtcgtgctccccggagtggaggcggccgagcgcgccggggtgcccgccttcctggagacctccgcgccccgcaacctccccttctacgagcggctcggcttcaccgtcaccgccgacgtcgaggtgcccgaaggaccgcgcacctggtgcatgacccgcaagcccggtgcctgataa

SEQ ID NO: 53 - DNA, 399 bp, synthetic construct
  source 1..399: mol_type = other DNA
atggccaagcctttgtctcaagaagaatccaccctcattgaaagagcaacggctacaatcaacagcatccccatctctgaagactacagcgtcgccagcgcagctctctctagcgacggccgcatcttcactggtgtcaatgtatatcattttactgggggaccttgtgcagaactcgtggtgctgggcactgctgctgctgcggcagctggcaacctgacttgtatcgtcgcgatcggaaatgagaacaggggcatcttgagcccctgcggacggtgccgacaggtgcttctcgatctgcatcctgggatcaaagccatagtgaaggacagtgatggacagccgacggcagttgggattcgtgaattgctgccctctggttatgtgtgggagggctaa

SEQ ID NO: 54 - DNA, 969 bp, synthetic construct
  source 1..969: mol_type = other DNA
agactagacggttcctggccttttgctggccttttgctcacatgtgagggcctatttcccatgattccttcatatttgcatatacgatacaaggctgttagagagataattggaattaatttgactgtaaacacaaagatattagtacaaaatacgtgacgtagaaagtaataatttcttgggtagtttgcagttttaaaattatgttttaaaatggactatcatatgcttaccgtaacttgaaagtatttcgatttcttggctttatatatcttgtggaaaggacgaaacaccgtgcgctcggcatgggtgcaatctctagggtgaaagtcccgaactgcgaaggcagaagtagcagttagcttaacgcaagggtgtccgtggtgacgcggaatctgaaggaagcgggcggcaaacttccggtctgaggaacacgaacttcatataaggctaggtatcattggatgagtttgcaagacaaaacaaagtcctttctgccgaaggtgatacagagtaaatgaagcagatagatggaaggaaagattgtactcttacccgaggaggtctgatggatacgtgaagtgcgcttcataacctacttagtgataagtaactgaaccatcagaagtcagcagaggtcatagtacgaatcggtctagaacgattcggaaggactgaacaatcaagagaaaatagcccttggcattcagtacgtcatgatgaacacagaaaacatggtacctcccaagagaaaggaaacggtgaatcccgtgggaatcttttggagggtggagtgacgactggcataagaagatcagctatttacggaaggaagcttgcgtcattatcttgattgaaccgccgtatacggaaccgtacgtacggtggtgtgagaggacggaggttaatcacctcctcctactcgatttttttttggtaccgacattgattattgactagtcatgtctg

SEQ ID NO: 55 - DNA, 957 bp, synthetic construct
  source 1..957: mol_type = other DNA
agactagacggttcctggccttttgctggccttttgctcacatgtgagggcctatttcccatgattccttcatatttgcatatacgatacaaggctgttagagagataattggaattaatttgactgtaaacacaaagatattagtacaaaatacgtgacgtagaaagtaataatttcttgggtagtttgcagttttaaaattatgttttaaaatggactatcatatgcttaccgtaacttgaaagtatttcgatttcttggctttatatatcttgtggaaaggacgaaacaccgtacgacgggcatgtcgtacatctgaggtgcaagtcctctgtggacacctgctaccggtgaacccaatagcgactcccaagcctgactatcgcgaggtaacggggagaggaagggatagcgaaatcgtggctctacgaacagaaacgtgatattaaggcgtatatagtggatgagggggctaggcactctaaagtccaaaaaggtagtcgtaatctatgtgcgtaaatcacgagagtaaacgaggaaagatgtacgacttatcccgtgaggtctcatgagcgtcaagtagacgtagtaataacgaatcatgagaagtcagccgaggtcatagtagtgatgaagtttctgtaatggaaacggagcgaaggaccgaacgattaaatgataccctatctaactgattttgtctgccctaacacctggtctgaaatgacggtactcgcagaacgtatgctgaaagaggctgctcacaaatataggacggcacaagcggaacgaaatcatatataggtaggtgtgggaacaaaaaaagtgttctcgccaaagtttagttgaaccgccgtgtgccgaacggcacgcacggtggtgtgagagggactatcaattagtccctactcgatttttttttggtaccgacattgattattgactagtcatgtctg

SEQ ID NO: 56 - RNA, 479 nt, synthetic construct
  source 1..479: mol_type = other RNA
  misc_feature 181..186: note = note = n=a, u, g, or c
gtgtgcccggcatgggtgcagtctatagggtgagagtcccgaactgtgaaggcagaagtaacagttagcctaacgcaagggtgtccgtggcgacatggaatctgaaggaagcggacggcaaaccttcggtctgaggaacacgaacttcatatgaggctaggtatcaatggatgagtttgcnnnnnnaaacaaagtcctttctgccaaagttggtacagagtaaatgaagcagattgatgaagggaaagactgcattcttacccggggaggtctgatcgaaacgccaagcactcttggtaacccattcagcaatggatggctgaacggtcagaagtcagcagaagtcatagtaccctgcatactcgagaatgtaaggggaaggacggaacaattaagttcgcttaattgaaccgccgtataccgaacggtacgtacggtggtgtgagaggacgggggttagtcgctcccttctactctat

SEQ ID NO: 57 - RNA, 479 nt, Oceanobacillus iheyensis
  source 1..479: mol_type = other RNA
gtgtgcccggcatgggtgcagtctatagggtgagagtcccgaactgtgaaggcagaagtaacagttagcctaacgcaagggtgtccgtggcgacatggaatctgaaggaagcggacggcaaaccttcggtctgaggaacacgaacttcatatgaggctaggtatcaatggatgagtttgcataacaaaacaaagtcctttctgccaaagttggtacagagtaaatgaagcagattgatgaagggaaagactgcattcttacccggggaggtctgatcgaaacgccaagcactcttggtaacccattcagcaatggatggctgaacggtcagaagtcagcagaagtcatagtaccctgcatactcgagaatgtaaggggaaggacggaacaattaagttcgcttaattgaaccgccgtataccgaacggtacgtacggtggtgtgagaggacgggggttagtcgctcccttctactctat

SEQ ID NO: 58 - DNA, 969 bp, synthetic construct
  source 1..969: mol_type = other DNA
agactagacggttcctggccttttgctggccttttgctcacatgtgagggcctatttcccatgattccttcatatttgcatatacgatacaaggctgttagagagataattggaattaatttgactgtaaacacaaagatattagtacaaaatacgtgacgtagaaagtaataatttcttgggtagtttgcagttttaaaattatgttttaaaatggactatcatatgcttaccgtaacttgaaagtatttcgatttcttggctttatatatcttgtggaaaggacgaaacaccgtgcgctcggcatgggtgcaatctctagggtgaaagtcccgaactgcgaaggcagaagtagcagttagcttaacgcaagggtgtccgtggtgacgcggaatctgaaggaagcgggcggcaaacttccggtctgaggaacacgaacttcatataaggctaggtatcattggatgagtttgctaaggtaaacaaagtcctttctgccgaaggtgatacagagtaaatgaagcagatagatggaaggaaagattgtactcttacccgaggaggtctgatggatacgtgaagtgcgcttcataacctacttagtgataagtaactgaaccatcagaagtcagcagaggtcatagtacgaatcggtctagaacgattcggaaggactgaacaatcaagagaaaatagcccttggcattcagtacgtcatgatgaacacagaaaacatggtacctcccaagagaaaggaaacggtgaatcccgtgggaatcttttggagggtggagtgacgactggcataagaagatcagctatttacggaaggaagcttgcgtcattatcttgattgaaccgccgtatacggaaccgtacgtacggtggtgtgagaggacggaggttaatcacctcctcctactcgatttttttttggtaccgacattgattattgactagtcatgtctg